European Patent Specification EP 3 789 506 B1, published October 18, 2023. Title: SNP MOLECULAR MARKERS FOR WEEPING TRAIT OF MEI AND USE THEREOF. Applicant: Beijing Forestry University. The sequence listing filed with the application follows.

SEQUENCE LISTING (14 sequences)

SEQ ID NO: 1 - DNA, 830 bp, Artificial Sequence
  Prunus mume
atgagtgcgagttaaagaatcgtggtggtaaatgattggctttctttggtcatgcttgagaaatctttaatgagtgtgagttgaagagtcctgatggtgtatgattgcctttacttggtgatggttgagaatggacaatgagcgtgagttgaatagtcttgatagtaaatgatttatttgtttggtcaatgacattgtggtttctaaaaacttgttcattgggttttagcaatccaccaatttggtggaagctttaagattctttggagtataaggaaccaaattgtagtttttgtttacactctggatattacactttggagttcctttcatatatgttctttgtgaaagtaaatcattgtgagaaaagaaattgattttgaccggtattattagtggttcatctggaatctgaatagatgccatttgatctctgttgcttatgaagtcagtgtttggtgtgcagctgccacttcctcaacagcagcagcagcagcttcggcagcaagagaatgcacttcctaagcagaggcctcaaacactcgatttgctctttgcaaacatgaaggagcaaaggatgagggcccaaccacgccagaacaatgccgtacctcgcaacattaggggtgtccagcagaggcccccttggggaagaggcggacgatttggcaactgattcatacgcataatgtgccagctagaaaggggattgaatgtctactttgtctagatcccaatgtgtagctgatgggggttcatatccaaaatatattggggccgtccgacttttgttgcctttatttttccatttttatgactttggaagactt

SEQ ID NO: 2 - DNA, 855 bp, Artificial Sequence
  Prunus mume
tcattatagaaacatgggaacatgagtaaaaataatttcccaagcttagggaatggtgtcgcttctagcaaagtacatcaagacaaacaactatatgatacaaacaaattcatctaaaataaaatctcaaaggctggaaccaaaaggccacaattataggcaactatatgcttggttcatctatcatgtatttttaatgtagaaaatatatccattcaactgtagaaccaactatatgaatggtttatctatcatgcttgatatatacttggtctcccccttcttgtttcttcaaggccttgctttatctgctttccactctcttctttctttcattggatctgagatcaaacaagatccatgaaattctgagttcaaaaaaaaaatcaaaatttagttattgtttcataacaaaaaaaattgaaatggaattagatacatttagaagtatcgataaaacaataacaacctttcaaagtaaaggctgtgaatgatgataagaataattcatggtgatataaggatatcaaatagctcaacatggataaatgctcaggccaaacttgactcacaagtcaaaccatgcttcattctccaactaaaccagaaaaagacaagaatacgtatgaatattaagtatatcaacaataataaatgattaaggcagatgtcatgtacttacttgggtgcctgctctgcacaagttcttacagagatgagaaaatggatgggatgtccatccaccatccacttagaaataatgaatttaacctcatagctcattttttgcttagtaacaagattatctttgttagaagtaataggattatgagctctcaattgaatatgccacat

SEQ ID NO: 3 - DNA, 20 bp, Artificial Sequence
  Prunus mume
tgagaatggacaatgagcgt

SEQ ID NO: 4 - DNA, 20 bp, Artificial Sequence
  Prunus mume
ctctgctggacacccctaat

SEQ ID NO: 5 - DNA, 20 bp, Artificial Sequence
  Prunus mume
cttagggaatggtgtcgctt

SEQ ID NO: 6 - DNA, 21 bp, Artificial Sequence
  Prunus mume
agagcaggcacccaagtaagt

SEQ ID NO: 7 - DNA, 21 bp, Artificial Sequence
  Prunus mume
tggaaactgaatagatgccat

SEQ ID NO: 8 - DNA, 21 bp, Artificial Sequence
  Prunus mume
tggaaactgaatagatgcgat

SEQ ID NO: 9 - DNA, 21 bp, Artificial Sequence
  Prunus mume
tggaaactgaatagatgcgaa

SEQ ID NO: 10 - DNA, 22 bp, Artificial Sequence
  Prunus mume
ggtgaaagagacatcagaaaat

SEQ ID NO: 11 - DNA, 23 bp, Artificial Sequence
  Prunus mume
catctaaaataaaatctcaaagg

SEQ ID NO: 12 - DNA, 23 bp, Artificial Sequence
  Prunus mume
tcataggtattcttgtctttttc

SEQ ID NO: 13 - DNA, 23 bp, Artificial Sequence
  Prunus mume
tcataggtattcttgtctttctc

SEQ ID NO: 14 - DNA, 23 bp, Artificial Sequence
  Prunus mume
tcataggtattcttgtctttctt